European Patent Application EP 4 339 205 A1, published March 20, 2024. Title: INDICATOR MOLECULE FOR TOXIGENICITY OF AFLATOXIGENIC FUNGI AND USE  THEREOF. Applicant: OIL CROPS RESEARCH INSTITUTE, CHINESE ACADEMY OF AGRICULTURAL SCIENCES. The sequence listing filed with the application follows.

SEQUENCE LISTING (1 sequence)

SEQ ID NO: 1 - protein, 33172 aa, Aspergillus flavus
AIGVEEPEADPTYYHNAIGVEEPEADPTYYHNNKAIGVEEPEADPTYYHNNKTTASMVWEEAQQVSGKASVETPASIEAASELSKAVSPSFEDVWSQPRDGAGQMFIPLNPNAYSPNTLNKDGAGQMFIPLNPNAYSPNTLNKGSPKDGVYVDKSVTSGFVDGIKDGLRDVGGPIEDQNSLQVGDRDVHGFATRFEQLPINQPRFGKPVGAVGSAAFGKPVGAVGSAATALKGDNEIPQAATAHDSAWDFFSQQPSGDNEIPQAATAHDSAWDFFSQQPSSLHGPNFEQLPINQPRGPTLLEDFIFRGVDFTEDPLLQGRGVGAHGVFTSYHGGPNFEQLPINQPRHVDGFGIHTFRLASVETPASIEAASELSKLFSYLDTQLNRLFYNSLTPAEQQFVVDAIRNAGIQTSRNAGIQTSRDGVYVDKNSLTPAEQQFVVDAIRNYFAETEQVMFQPGHNYFAETEQVMFQPGHIVRPEEYVPITKPLQIVIDGFRPNAYSPNTLNKPVGAVGSAATALKQDLFEAIEAGRQLSEDGVDVVVVAERSEDGVDVVVVAERSLTPAEQQFVVDAIRSMVWEEAQQVSGKSPSFEDVWSQPRSVETPASIEAASELSKSVTSGFVDGIKDGLRTTDVGTFGQKVDFTEDPLLQGRVETPASIEAASELSKVGFLASVETPASIEAASELSKYPEWELGVQIMDEEDQLKFDHERVPERFGFDLFDPTKFDLFDPTKFGKPVGAVGSAATNPDFMRQDLFEAIEAGRFVTDNGDSKLVKFVTDNGDSKSVTSGFVDGIKGFDLFDPTKVPVHNNNRDGAGQMFIPLNPNAYSPNTLNKIVPEEYVPITKDGVYVDKSVTSGFVDGIKFENSNVKSSVVRVGGPIEDQNSLQVGDRGDNEIPQAATAHDSVTSGFVDGIKDTTDVGTFGQKLKGVGAHGVFTGDNEIPQAATAHFVVDAIRTLLEDFIFRFTEDPLLQGRPDLIHAVKPRVDGFGIHTFRGVGAHGVFYLDTQLNRNVIIQLNRKPVGAVGSAATALKDGVYVDKNNVIIQLNRIVPEEYVPITKLGKTPAEQQFVVDAIRFENSNVKEQVMFQPGHIVRGVDFTEDPLLQGRAIGVEEPEADPTYYHNAIGVEEPEADPTYYHNASMVWEEAQQVSGKASMVWEEAQQVSGKASMVWEEAQQVSGKASMVWEEAQQVSGKASMVWEEAQQVSGKASMVWEEAQQVSGKASMVWEEAQQVSGKASMVWEEAQQVSGKASMVWEEAQQVSGKASMVWEEAQQVSGKASMVWEEAQQVSGKASMVWEEAQQVSGKASMVWEEAQQVSGKASMVWEEAQQVSGKASMVWEEAQQVSGKASMVWEEAQQVSGKASMVWEEAQQVSGKASMVWEEAQQVSGKASMVWEEAQQVSGKASMVWEEAQQVSGKASMVWEEAQQVSGKASMVWEEAQQVSGKASMVWEEAQQVSGKASMVWEEAQQVSGKASMVWEEAQQVSGKASMVWEEAQQVSGKASMVWEEAQQVSGKASMVWEEAQQVSGKAVSPSFEDVWSQPRAVSPSFEDVWSQPRAVSPSFEDVWSQPRAVSPSFEDVWSQPRAVSPSFEDVWSQPRAVSPSFEDVWSQPRAVSPSFEDVWSQPRAVSPSFEDVWSQPRAVSPSFEDVWSQPRAVSPSFEDVWSQPRAVSPSFEDVWSQPRAVSPSFEDVWSQPRAVSPSFEDVWSQPRAVSPSFEDVWSQPRAVSPSFEDVWSQPRAVSPSFEDVWSQPRAVSPSFEDVWSQPRAVSPSFEDVWSQPRAVSPSFEDVWSQPRAVSPSFEDVWSQPRAVSPSFEDVWSQPRAVSPSFEDVWSQPRAVSPSFEDVWSQPRAVSPSFEDVWSQPRAVSPSFEDVWSQPRAVSPSFEDVWSQPRDGAGQMFIPLNPNAYSPNTLNKDGAGQMFIPLNPNAYSPNTLNKDGAGQMFIPLNPNAYSPNTLNKDGAGQMFIPLNPNAYSPNTLNKDGAGQMFIPLNPNAYSPNTLNKDGAGQMFIPLNPNAYSPNTLNKDGAGQMFIPLNPNAYSPNTLNKGSPKDGAGQMFIPLNPNAYSPNTLNKGSPKDGVYVDKDGVYVDKDGVYVDKSVTSGFVDGIKDGVYVDKSVTSGFVDGIKFENSNVKSSVVRFGFDLFDPTKFGFDLFDPTKFGKPVGAVGSAATALKFGKPVGAVGSAATALKFGKPVGAVGSAATALKFGKPVGAVGSAATALKFGKPVGAVGSAATALKFGKPVGAVGSAATALKFGKPVGAVGSAATALKFGKPVGAVGSAATALKFGKPVGAVGSAATALKFGKPVGAVGSAATALKFGKPVGAVGSAATALKFGKPVGAVGSAATALKFGKPVGAVGSAATALKFVTDNGDSKFVTDNGDSKLVKFVTDNGDSKLVKFVTDNGDSKLVKGPTLLEDFIFRGVDFTEDPLLQGRGVDFTEDPLLQGRGVDFTEDPLLQGRGVDFTEDPLLQGRGVDFTEDPLLQGRGVDFTEDPLLQGRHGGPNFEQLPINQPRHGGPNFEQLPINQPRHGGPNFEQLPINQPRHGGPNFEQLPINQPRHGGPNFEQLPINQPRHGGPNFEQLPINQPRHGGPNFEQLPINQPRHGGPNFEQLPINQPRHGGPNFEQLPINQPRHGGPNFEQLPINQPRHGGPNFEQLPINQPRHGGPNFEQLPINQPRHGGPNFEQLPINQPRHGGPNFEQLPINQPRHGGPNFEQLPINQPRHGGPNFEQLPINQPRHGGPNFEQLPINQPRHGGPNFEQLPINQPRHGGPNFEQLPINQPRHGGPNFEQLPINQPRHGGPNFEQLPINQPRHGGPNFEQLPINQPRHGGPNFEQLPINQPRHVDGFGIHTFRHVDGFGIHTFRHVDGFGIHTFRHVDGFGIHTFRHVDGFGIHTFRHVDGFGIHTFRHVDGFGIHTFRHVDGFGIHTFRHVDGFGIHTFRHVDGFGIHTFRHVDGFGIHTFRHVDGFGIHTFRHVDGFGIHTFRHVDGFGIHTFRHVDGFGIHTFRHVDGFGIHTFRHVDGFGIHTFRHVDGFGIHTFRHVDGFGIHTFRHVDGFGIHTFRIVPEEYVPITKIVPEEYVPITKIVPEEYVPITKLFSYLDTQLNRLFSYLDTQLNRLFSYLDTQLNRLFSYLDTQLNRLFYNSLTPAEQQFVVDAIRLFYNSLTPAEQQFVVDAIRNAGIQTSRNAGIQTSRDGVYVDKNNVIIQLNRNYFAETEQVMFQPGHNYFAETEQVMFQPGHIVRNYFAETEQVMFQPGHIVRNYFAETEQVMFQPGHIVRNYFAETEQVMFQPGHIVRNYFAETEQVMFQPGHIVRNYFAETEQVMFQPGHIVRNYFAETEQVMFQPGHIVRNYFAETEQVMFQPGHIVRNYFAETEQVMFQPGHIVRNYFAETEQVMFQPGHIVRNYFAETEQVMFQPGHIVRNYFAETEQVMFQPGHIVRNYFAETEQVMFQPGHIVRNYFAETEQVMFQPGHIVRNYFAETEQVMFQPGHIVRQDLFEAIEAGRQDLFEAIEAGRQLSEDGVDVVVVAERQLSEDGVDVVVVAERQLSEDGVDVVVVAERQLSEDGVDVVVVAERSLQGKASMVWEEAQQVSGKSLQGKASMVWEEAQQVSGKSPSFEDVWSQPRSVTSGFVDGIKSVTSGFVDGIKDGLRSVTSGFVDGIKDGLRSVTSGFVDGIKDGLRSVTSGFVDGIKDGLRSVTSGFVDGIKDGLRSVTSGFVDGIKDGLRSVTSGFVDGIKDGLRSVTSGFVDGIKDGLRSVTSGFVDGIKDGLRSVTSGFVDGIKDGLRTTDVGTFGQKTTDVGTFGQKTTDVGTFGQKTTDVGTFGQKTTDVGTFGQKLKTTDVGTFGQKLKVGFLASVETPASIEAASELSKVGFLASVETPASIEAASELSKVGFLASVETPASIEAASELSKVGFLASVETPASIEAASELSKVGFLASVETPASIEAASELSKVGFLASVETPASIEAASELSKVPVHNNNRDGAGQMFIPLNPNAYSPNTLNKVPVHNNNRDGAGQMFIPLNPNAYSPNTLNKVPVHNNNRDGAGQMFIPLNPNAYSPNTLNKYPEWELGVQIMDEEDQLKYPEWELGVQIMDEEDQLKALFNRDIATGKANNYCSNQVEGPYSLYSGRDIATGKVSIAKDYACPWNGGEEVSLKDYACPWNGGEEVSLKVEYSDAAKEGDPEMYGNNETVNKVCAKANNYCSNQVEGPYSLYSGREPGICETTPGVKEQTASVVNGTAVIKGFSATGDYPRGGPGSSSMIGLMQENGPCRGYLEDIAYVLDSGIKGYYDISHFDPDIGLMQENGPCRLAAEGDPEMYGNNETVNKNAPLSIWMNGGPGSSSMIGLMQENGPCRNQVEGPYSLYSGRNYCSNQVEGPYSLYSGRPGGCKDQIIECRQVEGPYSLYSGRQYGNFSFTRSNQVEGPYSLYSGRTNASYVGGLVRTVYDMAMEAWSKTVYDMAMEAWSKPGGTVYDMAMEAWSKPGGCKVALVYGDRDYACPWNGGEEVSLKVFEAGHEVPAYQPETAYEIFVFEAGHEVPAYQPETAYEIFHRVSIWTESYGGRYCSNQVEGPYSLYSGRYGPSFTAFFQEQNEKVALVYGDRVEYSDAAKFRISYKEPGICETTPGVKFTAFFQEQNEKSIWTESYGGRNYIVVDADSSFWFFESRISYKEPGIHDDRVSIWTESYGGRYGPSFTAFFQEQNEKVALVYGDRDYAANNYCSNQVEGPYSLYSGRANNYCSNQVEGPYSLYSGRANNYCSNQVEGPYSLYSGRANNYCSNQVEGPYSLYSGRANNYCSNQVEGPYSLYSGRANNYCSNQVEGPYSLYSGRANNYCSNQVEGPYSLYSGRANNYCSNQVEGPYSLYSGRANNYCSNQVEGPYSLYSGRANNYCSNQVEGPYSLYSGRANNYCSNQVEGPYSLYSGRANNYCSNQVEGPYSLYSGRANNYCSNQVEGPYSLYSGRANNYCSNQVEGPYSLYSGRANNYCSNQVEGPYSLYSGRANNYCSNQVEGPYSLYSGRANNYCSNQVEGPYSLYSGRANNYCSNQVEGPYSLYSGRANNYCSNQVEGPYSLYSGRDIATGKVSIAKDYACPWNGGEEVSLKDYACPWNGGEEVSLKGDPEMYGNNETVNKVCAKANNYCSNQVEGPYSLYSGRGGPGSSSMIGLMQENGPCRIGLMQENGPCRIGLMQENGPCRISYKEPGICETTPGVKISYKEPGICETTPGVKISYKEPGICETTPGVKISYKEPGICETTPGVKISYKEPGICETTPGVKISYKEPGICETTPGVKISYKEPGICETTPGVKNAPLSIWMNGGPGSSSMIGLMQENGPCRNAPLSIWMNGGPGSSSMIGLMQENGPCRNAPLSIWMNGGPGSSSMIGLMQENGPCRNAPLSIWMNGGPGSSSMIGLMQENGPCRNAPLSIWMNGGPGSSSMIGLMQENGPCRNAPLSIWMNGGPGSSSMIGLMQENGPCRNAPLSIWMNGGPGSSSMIGLMQENGPCRNAPLSIWMNGGPGSSSMIGLMQENGPCRNAPLSIWMNGGPGSSSMIGLMQENGPCRNAPLSIWMNGGPGSSSMIGLMQENGPCRNAPLSIWMNGGPGSSSMIGLMQENGPCRPGGCKDQIIECRTVYDMAMEAWSKTVYDMAMEAWSKTVYDMAMEAWSKTVYDMAMEAWSKTVYDMAMEAWSKTVYDMAMEAWSKTVYDMAMEAWSKTVYDMAMEAWSKPGGTVYDMAMEAWSKPGGTVYDMAMEAWSKPGGCKTVYDMAMEAWSKPGGCKTVYDMAMEAWSKPGGCKTVYDMAMEAWSKPGGCKTVYDMAMEAWSKPGGCKTVYDMAMEAWSKPGGCKTVYDMAMEAWSKPGGCKTVYDMAMEAWSKPGGCKVALVYGDRDYACPWNGGEEVSLKVALVYGDRDYACPWNGGEEVSLKVALVYGDRDYACPWNGGEEVSLKVALVYGDRDYACPWNGGEEVSLKVALVYGDRDYACPWNGGEEVSLKVALVYGDRDYACPWNGGEEVSLKVALVYGDRDYACPWNGGEEVSLKVALVYGDRDYACPWNGGEEVSLKVALVYGDRDYACPWNGGEEVSLKVALVYGDRDYACPWNGGEEVSLKVFEAGHEVPAYQPETAYEIFHRVFEAGHEVPAYQPETAYEIFHRVFEAGHEVPAYQPETAYEIFHRVFEAGHEVPAYQPETAYEIFHRVFEAGHEVPAYQPETAYEIFHRVFEAGHEVPAYQPETAYEIFHRVFEAGHEVPAYQPETAYEIFHRVFEAGHEVPAYQPETAYEIFHRVFEAGHEVPAYQPETAYEIFHRVSIWTESYGGRVSIWTESYGGRVSIWTESYGGRVSIWTESYGGRVSIWTESYGGRVSIWTESYGGRVSIWTESYGGRVSIWTESYGGRVSIWTESYGGRVSIWTESYGGRVSIWTESYGGRVSIWTESYGGRYGPSFTAFFQEQNEKYGPSFTAFFQEQNEKYGPSFTAFFQEQNEKAAWLFEDSQAKADEINQIFDAISYMKADVPSGSTNITHGRAFPCFDEPALKAGMIADAGALASSGYQSTSGLLSLLKAVEQSLDAIRDGHILQQFKFAAGETSAIHPNIRGFDNEAEFIVWNEIVARIVDVLLDEKIVDVLLDEKNSGASRLNADHSAIYRLTFTGILNDNMAGFYRNGGEKEYNVVYDRNQDIYMPLGGLRNVGFPVVTVAEDAASSSIKSSHPIEVPVKSSHPIEVPVKRTGDVRPEEDTTLYPVMLGLRTHEIGWEFSEKTKQGLDENTMLTERTLGLALSDEVKVYATPDQDIEHGRYLASTQMEPTDARYLGEDVFIQGVRQGLLTVEDRGSVFSIVLKAAQEMFQRQGLDENTMLTERTDVESWLKAGMIADAGALASSGYQSTSGLLSLLKFAAGETSAIHPNIRLTFTGILNDNMAGFYRNGGEKEYNVVYDRNGGEKEYNVVYDRNGGEKEYNVVYDRNGGEKEYNVVYDRNQDIYMPLGGLRVYATPDQDIEHGRYLASTQMEPTDARAWYENGITNCVGDNTRCCDSGVEQLVSFSDVSDFKDADACNGGGIEYDSPADTPLEFKDNTCNAPIPVSFPVAPTDTKDPYMFHQANLRDQCNYSLQYTIGNKFAANGNYGSETTAAVINNFNGRFTTSASDGFDGMQVNPRGNGVIEAAAGKGNVAGNILVIAKITTADMDGISSWLPTINGKIYYNCDTPACTVQEWIDTSAGSGDFSNLLATEKKPLGTGTDLWPKLDDLFVWWTTPANRLVDWPIVTITHQEMSANMNAGSSYFVEVGHNMNAGSSYFVEVGHNGNGVIEAAAGKQAWVETMVQEFVRSMWPYFTTSASDGFDGMQVNPRTPLLNQQNSMWPYFTTSASDGFDGMQVNPRVIANGNVAGNILVIAKYFTSNGIIPPAITGLHNGDALRQITGVTLSAKSASDGFDGMQVNPRDPYMFHQANSDVSDFKEAGLKGIIPPAITGLHNGDALRYFTSNGIIPPAITGLHNEISFNQAWLRLVDWPIVTITHQEMSANFLDRKPLGTGTDLANGNVAGNILVIAKHQEMSANFLDRYNRDQCNYSLQYTIGNKAWYENGITNCVGDNTRAWYENGITNCVGDNTRAWYENGITNCVGDNTRAWYENGITNCVGDNTRAWYENGITNCVGDNTRAWYENGITNCVGDNTRAWYENGITNCVGDNTRAWYENGITNCVGDNTRDADACNGGGIEYDSPADTPLEFKDADACNGGGIEYDSPADTPLEFKDADACNGGGIEYDSPADTPLEFKDNTCNAPIPVSFPVAPTDTKDNTCNAPIPVSFPVAPTDTKDPYMFHQANDPYMFHQANLRDPYMFHQANLRDPYMFHQANLRDPYMFHQANLRDQCNYSLQYTIGNKEISFNQAWLREISFNQAWLREISFNQAWLREISFNQAWLREISFNQAWLREISFNQAWLREISFNQAWLRFAANGNYGSETTAAVINNFNGRFAANGNYGSETTAAVINNFNGRFAANGNYGSETTAAVINNFNGRFAANGNYGSETTAAVINNFNGRFAANGNYGSETTAAVINNFNGRFAANGNYGSETTAAVINNFNGRFAANGNYGSETTAAVINNFNGRFAANGNYGSETTAAVINNFNGRFAANGNYGSETTAAVINNFNGRITTADMDGISSWLPTINGKITTADMDGISSWLPTINGKITTADMDGISSWLPTINGKITTADMDGISSWLPTINGKITTADMDGISSWLPTINGKKPLGTGTDLWPKKPLGTGTDLWPKKPLGTGTDLWPKKPLGTGTDLWPKKPLGTGTDLWPKKPLGTGTDLWPKKPLGTGTDLWPKKPLGTGTDLWPKKPLGTGTDLWPKKPLGTGTDLWPKKPLGTGTDLWPKKPLGTGTDLWPKLDDLFVWWTTPANRLDDLFVWWTTPANRLDDLFVWWTTPANRLDDLFVWWTTPANRLVDWPIVTITHQEMSANLVDWPIVTITHQEMSANFLDRLVDWPIVTITHQEMSANFLDRMNAGSSYFVEVGHNGNGVIEAAAGKMNAGSSYFVEVGHNGNGVIEAAAGKMNAGSSYFVEVGHNGNGVIEAAAGKMNAGSSYFVEVGHNGNGVIEAAAGKMNAGSSYFVEVGHNGNGVIEAAAGKMNAGSSYFVEVGHNGNGVIEAAAGKMNAGSSYFVEVGHNGNGVIEAAAGKMNAGSSYFVEVGHNGNGVIEAAAGKMNAGSSYFVEVGHNGNGVIEAAAGKTPLLNQQNSMWPYFTTSASDGFDGMQVNPRTPLLNQQNSMWPYFTTSASDGFDGMQVNPRTPLLNQQNSMWPYFTTSASDGFDGMQVNPRTPLLNQQNSMWPYFTTSASDGFDGMQVNPRTPLLNQQNSMWPYFTTSASDGFDGMQVNPRTPLLNQQNSMWPYFTTSASDGFDGMQVNPRTPLLNQQNSMWPYFTTSASDGFDGMQVNPRVIANGNVAGNILVIAKVIANGNVAGNILVIAKYFTSNGIIPPAITGLHNGDALRASHTVDKNGIWSSEVKATDNYIANAAAAVAKDLLQDIVTWDDKEAGIYLIARGPLNEGGLYAERGTNYVALSLWALESDGAKHTDYSSQESTSYKLGSFELSYTTPVLTGYGNVESPEQPKLSGQDASAITWKLTGNLGGEDYQDKLTGNLGGEDYQDKVRNSAYNYWVPELPTEGTSPGFSTSKPGIGFYTAQFDLDLPKQGFHQPQPPSESWESGSPLEGLSKSPGSFFVVRSSYDDSAWVSADLPKTSYDYGSPITETRYPDADYMQYVMDQARNGIWSSEVKVLVLYGGPKASPSYLTATPRYLDTLPEIKTLHLEQSPSTPYAQLYVNGYQYGKKADIVVPFPWGGPGFEKAQLYVNGYQYGKAQLYVNGYQYGKATDNYIANAAAAVAKLSGQDASAITWKLTGNLGGEDYQDKVRNGIWSSEVKQGFHQPQPPSESWESGSPLEGLSKSSYDDSAWVSADLPKYPDADYMQYVMDQARYPDADYMQYVMDQARALTNGAGAIKEAIADVLEHLGENDEDIAVYAPNPFYKGFAPLEYLGSNFENGELPKGFDNAGFVMGTSSSLFNQFILRGKMPMPILVADGRHFQLINTAAYWKIPNVAIAVSGGGYRLNGTDIPNFLKLNLSSFDASGYIDRLPDICNTCFKMPMPILVADGRNSILEGPDVKSAAALSTSEKDWLQVRSSSLFNQFILRTFLNLGLNKTNTKLPDICNTCFKTSLTDYWGRSSFDASGYIDRSTSEKDWLQVRGTDIPNFLKLNLGLNKGFDNAGFVMGTSSSLFNQFEYLGSNFENGELPKMPILVADGRDLYDAVKINTAAYWKSIALGDDFKKALTNGAGAIKALTNGAGAIKALTNGAGAIKALTNGAGAIKGKMPMPILVADGRGKMPMPILVADGRGKMPMPILVADGRGKMPMPILVADGRGKMPMPILVADGRGKMPMPILVADGRHFQLINTAAYWKHFQLINTAAYWKLPDICNTCFKLPDICNTCFKMPILVADGRMPMPILVADGRMPMPILVADGRMPMPILVADGRMPMPILVADGRMPMPILVADGRMPMPILVADGRMPMPILVADGRMPMPILVADGRMPMPILVADGRNSILEGPDVKNSILEGPDVKNSILEGPDVKSAAALSTSEKDWLQVRSAAALSTSEKDWLQVRSAAALSTSEKDWLQVRSAAALSTSEKDWLQVRSAAALSTSEKDWLQVRSAAALSTSEKDWLQVRSAAALSTSEKDWLQVRSAAALSTSEKDWLQVRSAAALSTSEKDWLQVRSAAALSTSEKDWLQVRSAAALSTSEKDWLQVRSAAALSTSEKDWLQVRSAAALSTSEKDWLQVRSAAALSTSEKDWLQVRSAAALSTSEKDWLQVRSAAALSTSEKDWLQVRSAAALSTSEKDWLQVRSAAALSTSEKDWLQVRSAAALSTSEKDWLQVRSAAALSTSEKDWLQVRSAAALSTSEKDWLQVRSAAALSTSEKDWLQVRSAAALSTSEKDWLQVRSAAALSTSEKDWLQVRSAAALSTSEKDWLQVRSAAALSTSEKDWLQVRTNTKLPDICNTCFKTNTKLPDICNTCFKTNTKLPDICNTCFKAASLPASFSGFKALVSHDGTFVADAKENSLVWHQQVLGWLNKFNAVFSGTLKGDAGSPVFSPDSKGDAGSPVFSPDSKKIAYWQMADESYEADHRIQAFVIYPENFDKLFSIPADAGDDYKPKLNPEGLISAPRLPVSEGLSLFNILQERMINWIQGSDLGRNAESPYPPFGGASDYDLSPDGKRSEAIPNPSGDVAVFSQSQYSFKSEAIPNPSGDVAVFSQSQYSFKTAVPINGPDSPGTPEGVKTAVPINGPDSPGTPEGVKGDAGSPVFSPDSKTLATANKIDPELKTLYVYTVGSEETIPSLAADWDRTTSQWNVLDLKVVTTDSGDVRWIQGSDLGRALVSHDGTFVADAKALVSHDGTFVADAKGDAGSPVFSPDSKKIAYWQMADESYEADHRIAYWQMADESYEADHRIAYWQMADESYEADHRLFSIPADAGDDYKPKLFSIPADAGDDYKPKLNPEGLISAPRRSEAIPNPSGDVAVFSQSQYSFKRSEAIPNPSGDVAVFSQSQYSFKTAVPINGPDSPGTPEGVKTAVPINGPDSPGTPEGVKTAVPINGPDSPGTPEGVKGDAGSPVFSPDSKTTSQWNVLDLKTTSQWNVLDLKAASNFDGDTLVLGYDSGNGNPETSFMTLMRAGSTIAVTDVQITGGAVGIKASGTCSGPIQSAPTSYWLADQDHSGDARDAGSPKPVVQIGHEGDVGVAEIQNMRFSVAEILPGAKGDGSTDDSASLNAILANNAANCKGTCSGPIQSAPTSYWLADQDHSGDARIVGEAWAVITGAGDAFKNSQILIQNLSHDNSNAIAVDSKNSQILIQNLSHDNSNAIAVDSKDNIKNVVLDTTALSANTKSAPTSYWLADQDHSGDARVGTIITGDPLDPPVLKVTNSPSNLVWYSISTRYPAEVFLPGGTYQLGKSLGSLVLLDSSSINSGPVVRDTLVIPPGSRAQPTYAEYSNDQIVNVKSGTCSGPIQSAPTSYWLADQDHSGDARAGSTIAVTDVQITGGAVGIKAQPTYAEYSNDQIVNVKAQPTYAEYSNDQIVNVKDAGSPKPVVQIGHEGDVGVAEIQNMRFSVAEILPGAKNSQILIQNLSHDNSNAIAVDSKNSQILIQNLSHDNSNAIAVDSKNSQILIQNLSHDNSNAIAVDSKNSQILIQNLSHDNSNAIAVDSKDNIKNSQILIQNLSHDNSNAIAVDSKDNIKNSQILIQNLSHDNSNAIAVDSKDNIKNVVLDTTALSANTKSAPTSYWLADQDHSGDARVTNSPSNLVWYSISTRVTNSPSNLVWYSISTRAGALLLGKAGVIPESLHQDTVGTFGKDRLETTAGSWALLGSVVPRGIMDETYYQALEFCQRGKTPEGGYAQFLTNKGPLHGIPFIVKIHQTQPYLNAILQVNPDAFKLETTAGSWALLGSVVPRNSVVGIKPTVGLTSRTIVSPDGFNWDYGSTRTPEGGYAQFLTNKTTREEGIDAALKVDFYNNLKDYLSEVENTKAALSEWADMRALGTETDGSVINPAQREEGIDAALKDAVYALDAIYGIDARAALSEWADMRAALSEWADMRAGVIPESLHQDTVGTFGKAGVIPESLHQDTVGTFGKAGVIPESLHQDTVGTFGKAGVIPESLHQDTVGTFGKGIMDETYYQALEFCQRIHQTQPYLNAILQVNPDAFKNSVVGIKPTVGLTSRNSVVGIKPTVGLTSRNSVVGIKPTVGLTSRTIVSPDGFNWDYGSTRTTREEGIDAALKAVWPGDMGVAVPAAFVSTGDLESVKAYQGYFHSNDDLLNRDGSASYVMPDKDRAVWPGDMGVAVPAAFVSTGDLESVKDSAFPGLWEENIYAPSSRGGSGALGLAFSEAKGVYYVDDTATITVSGGGSHRIWYSGAYTLQTNAVPVNTGRNALQTMYDTQDKNALQTMYDTQDKTTGAFDESGPPLSQKSPDGYTLQFSVPPGTKSSEKPSITIDGNNINKTTGAFDESGPPLSQKIAPQFGDLKALELIRRFQASWDKSPDGYTLQFSVPPGTKISSFEIQGHFKAVWPGDMGVAVPAAFVSTGDLESVKAYQGYFHSNDDLLNRAYQGYFHSNDDLLNRAYQGYFHSNDDLLNRAYQGYFHSNDDLLNRDGSASYVMPDKDGSASYVMPDKDRAVWPGDMGVAVPAAFVSTGDLESVKGVYYVDDTATITVSGGGSHRGVYYVDDTATITVSGGGSHRISSFEIQGHFKNALQTMYDTQDKNALQTMYDTQDKNALQTMYDTQDKNALQTMYDTQDKTTGAFDESGPPLSQKNALQTMYDTQDKTTGAFDESGPPLSQKNALQTMYDTQDKTTGAFDESGPPLSQKNALQTMYDTQDKTTGAFDESGPPLSQKSPDGYTLQFSVPPGTKSPDGYTLQFSVPPGTKSSEKPSITIDGNNINKSSEKPSITIDGNNINKSSEKPSITIDGNNINKTTGAFDESGPPLSQKDNILPENLDDGLPSQFVYEKFGPHEYNGDQYTSIIRLVIDLSGNGGGYILQGYDTFRNVGLVSVSLDGKPSSDPMQGIGGIKQLFPSIVQDGYTRSDKYAGEYEFQADLFKSFEPSTPAEFQAVLEKYAGEYEFQADLFKPFAASTPGFDGYFSGSARAASTPGFDGYFSGSARYDLNLENKAFNLAHDGHFRHFTSLEEKFFPDLLTKSIAIGGRPSSDPMQGIGGIKFGPHEYNGDQYTSIIRFGPHEYNGDQYTSIIRQLFPSIVQDGYTRQLFPSIVQDGYTRQLFPSIVQDGYTRSDKYAGEYEFQADLFKEPGAEGVCETTPGVKFANQMPNGCQDLISTCKGCQDLISTCKQLPKNPTGVKSAGYTPLKVNGVEYGETRSYSGYVDTSPESHTFTALADYALCAEATNMCRTIFGWDIAEGQKTIFGWDIAEGQKKVYEAGHEVPYYQPIASLYKEPGAEGVCETTPGVKLSGLPSLDSRSYSGYVDTSPESHTFFHNPETAPITLWLNKIWPSYKVYEAGHEVPYYQPIASVNGVEYGETRTALADYALCAEATNMCAEGVCETTPGVKFANQMPNGCQDLISTCKFANQMPNGCQDLISTCKFANQMPNGCQDLISTCKFANQMPNGCQDLISTCKFANQMPNGCQDLISTCKFANQMPNGCQDLISTCKKIWPSYKKIWPSYKSAGYTPLKVNGVEYGETRSAGYTPLKVNGVEYGETRSAGYTPLKVNGVEYGETRSAGYTPLKVNGVEYGETRSAGYTPLKVNGVEYGETRSAGYTPLKVNGVEYGETRSAGYTPLKVNGVEYGETRSAGYTPLKVNGVEYGETRSAGYTPLKVNGVEYGETRSAGYTPLKVNGVEYGETRSAGYTPLKVNGVEYGETRTALADYALCAEATNMCRTALADYALCAEATNMCRTALADYALCAEATNMCRTALADYALCAEATNMCRTALADYALCAEATNMCRTALADYALCAEATNMCRTALADYALCAEATNMCRTALADYALCAEATNMCRTALADYALCAEATNMCRTIFGWDIAEGQKTIFGWDIAEGQKTIFGWDIAEGQKTIFGWDIAEGQKTIFGWDIAEGQKTIFGWDIAEGQKTIFGWDIAEGQKTIFGWDIAEGQKTIFGWDIAEGQKTIFGWDIAEGQKTIFGWDIAEGQKTIFGWDIAEGQKTIFGWDIAEGQKKVNGVEYGETRVNGVEYGETRVNGVEYGETRYKEPGAEGVCETTPGVKYKEPGAEGVCETTPGVKYKEPGAEGVCETTPGVKYKEPGAEGVCETTPGVKYKEPGAEGVCETTPGVKASDFWANELVTWWNKEAEPSQEYVSYSHGVFLRFSYEEGEKFLNKGAKDDVFIKGGSILPMQEVALTTRKATGDVLFNTKNAHGQEILLRNHNVLSAIPQEPYRQYQLSTVGLPAMQQYNTLGFHQCRSSEAEPSQEYVSYSHGVFLRTLGGSVDLTFYSGPTQAEVTKWASVIDATKSEAEPSQEYVSYSHGVFLRAEPSQEYVSYSHGVFLRAEPSQEYVSYSHGVFLRAEPSQEYVSYSHGVFLRAEPSQEYVSYSHGVFLRASDFWANELVTWWNKEAEPSQEYVSYSHGVFLREAEPSQEYVSYSHGVFLREAEPSQEYVSYSHGVFLRFSYEEGEKFLNKGGSILPMQEVALTTRGGSILPMQEVALTTRNAHGQEILLRNAHGQEILLRNHNVLSAIPQEPYRNHNVLSAIPQEPYRNHNVLSAIPQEPYRNHNVLSAIPQEPYRNHNVLSAIPQEPYRSEAEPSQEYVSYSHGVFLRWASVIDATKWASVIDATKDPSINDDSVMIYAPAVRFLDEALTYPPPKGIQINDPSINDDSVMIYAPAVRIASAMLDEEDEKYFNVKNGDQSPPSALGPLPSVIERPSINDDSVMIYAPAVRTDYSVCGETTIFKVYLTGESYAGQYIPYIASAMLDEEDEKVYLTGESYAGQYIPYIASAMLDEEDEKYFNVKIASAMLDEEDEKTDYSVCGETTIFKNGDQSPPSALGPLPSVIERVYLTGESYAGQYIPYTLIAGAGLLGTAHTERETTIFKNGDQSPPSALGPLPSVIERTDVQKALHVPRDDSVMIYAPAVRFLDEALTYPPPKGIQINDPSINDDSVMIYAPAVRGIQINDPSINDDSVMIYAPAVRGIQINDPSINDDSVMIYAPAVRGIQINDPSINDDSVMIYAPAVRIASAMLDEEDEKIASAMLDEEDEKYFNVKIASAMLDEEDEKYFNVKIASAMLDEEDEKYFNVKIASAMLDEEDEKYFNVKIASAMLDEEDEKYFNVKIASAMLDEEDEKYFNVKIASAMLDEEDEKYFNVKNGDQSPPSALGPLPSVIERTDYSVCGETTIFKNGDQSPPSALGPLPSVIERTDYSVCGETTIFKNGDQSPPSALGPLPSVIERVYLTGESYAGQYIPYIASAMLDEEDEKYFNVKAHILPPNGRDLNPNGSQFITPGGKDLNPNGSQFITPGGKNDPVAVFDGSVIPKEAGLVPFQVSPTTKFHVLTAQLSFPRFRDLNPNGSQFITPGGKLDRPPVIPLPPSDSDVTAFRNDPVAVFDGSVIPKPVAVFDGSVIPKTISNVVDNELARTTNGIVSTNESGRDPVAVFDGSVIPKFALSTWARILPATSQVSTKAHILPPNGRAHILPPNGRAHILPPNGRDLNPNGSQFITPGGKFALSTWARFALSTWARFHVLTAQLSFPRFHVLTAQLSFPRFRDLNPNGSQFITPGGKFRDLNPNGSQFITPGGKFRDLNPNGSQFITPGGKNDPVAVFDGSVIPKTISNVVDNELARTISNVVDNELARTISNVVDNELARTTNGIVSTNESGRDWSDSYYQGPAFKFGLGADNTLAFEVVTADGQLVTASRGVGSDAWTVSESGRITNEYVPQLEAVTPGSGCYQNEGNFRNVLENNPTGMASVLRSKWDPNNFFYVLKTTALTDLGIAYKVSAGVMGYQILNAAHAKVSYTEYDSYYDHYNKYMGPLPYGNLAVATYQYGGRWDPNNFFYVLKDWSDSYYQGPAFKGVGSDAWTVSESGRGVGSDAWTVSESGRGVGSDAWTVSESGRGVGSDAWTVSESGRITNEYVPQLEAVTPGSGCYQNEGNFRNVLENNPTGMASVLRNVLENNPTGMASVLRVSAGVMGYQILNAAHAKVSAGVMGYQILNAAHAKVSAGVMGYQILNAAHAKVSAGVMGYQILNAAHAKVSAGVMGYQILNAAHAKVSAGVMGYQILNAAHAKVSAGVMGYQILNAAHAKVSYTEYDSYYDHYNKYMGPLPYGNLAVATYQYGGRALMNGAGAIKDAGYETSITDYWGRDFFNHVTIKDGNWTTCVGCAILSRGFVPLEYVGSKHVYDAVQDKPTVYGFVPLEYVGSKTNTQVPDACTQCFQKQADMPMPLLVADGRTAFSDILAKSIALTDTFKILDSATYYKALMNGAGAIKALMNGAGAIKALMNGAGAIKALMNGAGAIKALMNGAGAIKALMNGAGAIKALMNGAGAIKALMNGAGAIKALMNGAGAIKDAGYETSITDYWGRDAGYETSITDYWGRDAGYETSITDYWGRDAGYETSITDYWGRDAGYETSITDYWGRDFFNHVTIKDFFNHVTIKDFFNHVTIKDFFNHVTIKGFDNAGFVMGTSSSLFNQFMPLLVADGRMPLLVADGRMPMPLLVADGRMPMPLLVADGRMPMPLLVADGRMPMPLLVADGRMPMPLLVADGRMPMPLLVADGRMPMPLLVADGRQADMPMPLLVADGRQADMPMPLLVADGRQADMPMPLLVADGRQADMPMPLLVADGRTSITDYWGRAHDDTVNYLYEELKKATAFAVATYANDLSSIPKGGDPNNVVALGGHTDSVEAGPGINDDGSGIISNLVIAKGPYSAIVGISLEDGQKNLGCSEADYPSDVEGKQPQVHLWSNADQTLKTMTYSPSVEVTADVAVVKTTYNVVAQTKVGDEEIEAKAHDDTVNYLYEELKKAHDDTVNYLYEELKKAHDDTVNYLYEELKKQPQVHLWSNADQTLKTMTYSPSVEVTADVAVVKAGQFPISANDGATSTKAGVLSWSYTWSPADKEAASAALAAGYKFDGVTWDEENWLLKFDPSAAIYPWTSGRFVGGASTDAFADPKLLPEEGIYITPNLPPQIPYVKPSAAIYPWTSGRVVLTLTGIEPSTIYTAEEENQVRAYVASDSELEYVTWTVDNRGDWEVTSILSIDQERTLIPADKIPTGKTLSTNEEGYETSAVRVSQTNPTVTLSLLNIASKYPILFTPYGGPGAQEVTKDGTDGWLDNLLSMKTLSTNEEGYETSAVRKFYDSMYTERTLIPADKIPTGKATSGGTSAAAPVFAGLVGMLNDARDFTDITAGSSIGCDGVNPQTGKGFPDVAAHSLTPRPDVAAHSLTPRPNSALPQVLSNSYGDEEQTVPEYYAKSALPQVLSNSYGDEEQTVPEYYAKSYGDEEQTVPEYYAKVCNLIGLMGLRLKDLVLSLAWYQESAVSKATSGGTSAAAPVFAGLVGMLNDARATSGGTSAAAPVFAGLVGMLNDARAWYQESAVSKAWYQESAVSKDFTDITAGSSIGCDGVNPQTGKGFPDVAAHSLTPRGFPDVAAHSLTPRGFPDVAAHSLTPRSALPQVLSNSYGDEEQTVPEYYAKVCNLIGLMGLRDAEEEPYDWSNEGRGISDGIDWQAGYSAVQKMDDAEQYEATSRNIYIQSATLDGKPYSKSLNYIPVEDFDYKTLEYSYDDFTIAQMARTMINPQDYTGENPLWKDNGIFVNSRSINGYPLPGGAFVRMDDAEQYEATSRTLEYSYDDFTIAQMARDIDFGENGDGIKDYVPNTQIPVTVAANTFPGGQEGFIDFVKFQESPEGADFWGARTKVTISPELSIRVFQTAFGPAGTMLTYEPIVRADAIVAAIRLAEDHINWVEIRVTISPELSIRHELGVDEIWRDIDFGENGDGIKDIDFGENGDGIKFQESPEGADFWGARLAEDHINWVEIRAGVKPSNYVGDIFGTLGGTPDFGPGRCDVATTDVYYSGKSKYTAEGYEAATKTASNFDQPHSDESALQHLRYCASAQEDNATLQALLRYTAEGYEAATKYVDAGGFEPSIKLQALLRSKYTAEGYEAATKTASNFDQPHSDESALQHLRGHLTAMTGDGVNDAPSLKTAALVQGASDSGHFKTGTLTANQLSIRAYGIVVATAKTGDGVNDAPSLKMLTGDALAIAKLAIEHEVDAHGKIENMLSHLSKDKSETETETEIEISNKIKEIQEAGDVRLSDELEDDNAPIGFETTKSVEIAQLHSEVEALVEKYTVTAGELTSDFKEVEVEKEWTKTETKTEIEIERIKEIQEAGDVRASSDDSNYGWEDSKGIQDAGVIATAKIGAQSTVLLKNFGEIGDASEYVYPEGLERYTPPNFSSWTRVNEFVDVQRAVDIVSQMTLTEKDSPNWDVDSDALPAIPEGAKEIPVGYSAADIDTNRGVDYQPGGSSNLADPIADAEGCKRNTLAFFSGNEVINDGPSSKYGLVEIDDGKVKTLADFDALKYGLVEIDDGKVKDLMQAMADFGPKFPGGNNLEGDTLDGRTGEVYASAVIVSKYPSNLDAWIPVDGSALSLKYVEVGNEDNLNDGLDSYKFQAFYDAIKEQTYTGSFYVKASLGHPEPWTVKDLMQAMADFGPKELPSGPYFVSLYTGEVFKGISPEAHQSLTTFTRLYPDDNLAFIQAGISDEKQLLLAGGGWDGKSLFVSVYSVGTTDYRLYYTPTAEKPLAGLRGISPEAHQSLTTFTRQLLLAGGGWDGKDSLSEAIAYAKGGGGGTFGVVMESTHRIANECQNQELFWALRSQGGTAVIEEFPSWYEFYQKYVVPNAVTVGNAHFAATRSSGQGTLSLWTRAVTVGNAHFAATRGGGGGTFGVVMESTHRGGGGGTFGVVMESTHRGGGGGTFGVVMESTHRIANECQNQELFWALRSSGQGTLSLWTRYVVPNAVTVGNAHFAATRYVVPNAVTVGNAHFAATRYVVPNAVTVGNAHFAATRASSVSGVITLSDGRTTADSDGNFSFENVRVQDETWELSDGSYITKYDWSDFINSAKYEEFEVPAGTLVKIWQIGTLDRAYTQYTETSVYGMLKDGDLVTQQNELQGKHEGWIDEAAVQEAKLHYGAYSIKSNLFNSYSENQVLLPASVYGSYKETYGSAAGWDKLADALAASSLPEAWWGENYEPLLNIKGGGGGTFGVVIESTHRIANECQNQDLFWALRVEPQLSFVAAVIKYVTSNAVSVGVTHFAGSRAVFETAEGRGGGGGTFGVVIESTHRYVTSNAVSVGVTHFAGSRDAEVAPPNDPVDPMAPDSSTKFEGYLPDARGSTGNVLVDVSHVLPSFRVGISWLSTEKLSITATGGDGNGDSQIYVQKGAVNWEDGYRDAEVAPPNDPVDPMAPDSSTKDSVKEDDYEDLFNYICAKKFTDTPVLYGPKMLDDAGIYLITDLSSPSESINRSDGQCSDLLKQQLSFVMNQWYEKYGAYSVCSPKTLPAIESKKFTDTPVLYGPKMLDDAGIYLITDLSSPSESINRSDGQCSDLLKADAAGSHGEALNEVQAKAKADAAGSHGEALNEVQAKLEAAEQALSEARVGALESQLSTEQDAIKEAAESAGTTHSQQLQELRDALEAAEAAAKIQEQLKGQTPLPILVADGRNNILEGPDVKSHLSVVDGGEDGQNIPLHPLIQPERTIDYWTELVDTVKTSTTLPEVCSKAMLNGAGALKAMLNGAGALKAMLNGAGALKAMLNGAGALKAMLNGAGALKGQTPLPILVADGRINLGLNKNNILEGPDVKSHLSVVDGGEDGQNIPLHPLIQPERTFINLGLNKTSLTDYWGRFNVDETAFTGAWGRIGSLAITDVSLPFFKIQGISNPSGALSSGGLGEPKVQNGAVTWESDPNRATTVYGESIKSIYAINSGRELDTQHIHPPDSYFVSPLTRGFTEIDELWNGVTAETNAAQDLRQAQVAHDFWQKFYHQVVELNRKDAELTDAGVKLNTGAVIPVLVRELDTQHIHPPDSYFVSPLTRLNTGAVIPVLVRLNTGAVIPVLVRQAQVAHDFWQKQAQVAHDFWQKAINDYIDSQLDKKGVQISTNIPKSSPWIMLGGSYPGMRYQSLEYQQSLCYRLFSLALKISIPIDHEDPSMGTYQNRAINDYIDSQLDKKCSSHDDCSDELACTDGVCACTADSAVTCSWEGHCAGAKLNLQYQASGDAKKSLVDFSAARGDNPSILGLRSAVTCSWEGHCAGAKIGTTIDDIKCTADSAVTCSWEGHCAGAKCTADSAVTCSWEGHCAGAKCTADSAVTCSWEGHCAGAKCTADSAVTCSWEGHCAGAKAFPDVAAQGMNFAVYDKELYNIGDYQADANSGSKIAFASYLEEYARQGLQDITLGASIGCTGRYADLENFENYLAPWAKAFPDVAAQGMNFAVYDKAFPDVAAQGMNFAVYDKELYNIGDYQADANSGSKYADLENFENYLAPWAKYADLENFENYLAPWAKAGSSPTDIISGISDKTDALDSAIKKVEQAIDDIIAKSAADGLASAITSKSGDDISTTDALALPEPVQALTKSPTDIISGISDKTDALDSAIKAQNDPNAFGVVAARLGACPPGKETALLGDKPNAFGVVAARQNDPNAFGVVAARAATYCPENIEKIENQSDADGYSSCSTLKLTGLTTLTTLSFAALTKSDKLNVIDFPKVGSIEFTALPQLQSLDFTKLNVIDFPKTVNGGFQIARGVAAWLFERLSFGSIDLENANINRSLSFIPGVLYDGSPIGKQESTFAAVERSCFEIGKFVDPLIGSNNGGNVFAGASLPYGMAKGWTQGGSNADVVLTDAYVKVGISYISTDRAGNWQNLYKAQHPFLTIVDPEAQSRSVFSQNESVAAGLKTTAVLFDEGKEICLAALGRALVIVSDSIRTDTIHGVGQNSFYKASHPIEVPVKASHPIEVPVKIMSILLGGAIPDDLKPLVLFDSVTKTATESEPSLSDIEKTGYVNYNVDTTNLRKHNPLVLFDSVTKTSPFPYDSKKHNPLVLFDSVTKKHNPLVLFDSVTKKHNPLVLFDSVTKTGYVNYNVDTTNLRAPTPPDFSLGYIQSKIEQDGSESLLTNEYAPLKGYAFIWNMPAQGRTSGWGGNPGGYRYQLASYLRDYLDEYLVFPPAGVQPQKIYVTGESYAGRVDHLPDVPFDVGEMYSGLVPIDKDDKNFQELFGIKKTPLDDFRADDVLEVNPLADPEVVSYFRLDADAITAQYFGNDAPWYRSDYASFLYGPYRLVFAPQEEKATWDGVDADKIRFQYPGDLFDQGTTIRFTGDAATVNSIAARPDSDEIYFGGQFEKNLEVLSLTKHVAAYSFGSKAWTALGGGVNGPVHKNLALLDGKDLTDYLMKSYELPDGQVITIGNERVAPEEHPVLLTEAPINPKQEYDESGPSIVHRQEYDESGPSIVHRVAPEEHPVLLTEAPINPKVAPEEHPVLLTEAPINPKVAPEEHPVLLTEAPINPKAELPEGYPESSANPAFRDIQYLENYQGQGYSGPAVKFVTVTEETDPDLFWALRLSLGDSGACKDAEVEPANWGVEGRLGGAQLFTSRTVSLVEDGSNTPATLSAGTFARSLVDIYRTVSLVEDGSNTPATLSAGTFARAYVEMMQCTDEKEPLVRLEKDLPGTTLSSKYYGYGGGNPLGPAQGIGFANELIARLEKDLPGTTLSSKLSEAGHSVLLIEKTPIESDATSYLNDRGGPMGTYLVSASERVILSAGTFGTPKAVITDIVNQQRLINQVELSEDKTIARGGSNNFGIVTRLLLSDAMWYTRERPSAQLLSGKFDTLGTSGPTAKLANAYTWEGGRAVADRIPLAIHDEVSPVGDTDALLERAPVVQYALNRDGYMGYHGVPQIPIYAYKAIHDEVSPVGDTDALLERAIHDEVSPVGDTDALLERAIHDEVSPVGDTDALLERDGYMGYHGVPQIPIYAYKLAEESAALGVKVNPIILTGDMWRVSDNAGLGDWVPNPDRFPDGLTPLVEDVTKALGGTSTINGMAYTRSQLSDYAAATVKAEDVQIDVWQKALGGTSTINGMAYTREIGFTVQEDNTDGKIDFGSAPNIVNAIAEDRNSPVWPDGIQQTYEYPNRASTNMITSNSGAGLVPQDENRIGGSAGTELQSDKITGEVWPVLMAYGQKSAISQYGDSFAKSQSDFESEFSTAKVNAGIGIGPDDLVSFIKGNAMDHFSSIMERYGPTYAAYFLDQNEKAITETQYEEAKDLTLDLPDIGLQYAGTVKTVAALINWRNIWDGTTAQNVKKEDLETSSYSFSGDGKVDFASLQSAATQSTTYSNAPAVKTCSLVFLFPKKEDLETSSYSFSGDGKFDGILGLGFDTISVNKYGSGSLSGFVSQDTLKWYSVYDLGNGAVGLAKDAYSPHEIYSRIFEQLEGMSLSKTYEVVGNVYKDQVLKDVALIKAVPGTAQQAAAIKDAGEFDVERGTVVTNDQCGGASSVRLHLVTAEEADIKIIYDMPDGSSCKGIDVAKPTGRVNGVWTVTHSPFEGLSALKSAMTLPRVNGVWTVTHSPFEGLSALKVPTVLMSPWVGKSIDQFFNDAKNVAPDDPDHSITGGNQQVYSTYHPNAKESTLHLVLRIQDKEGIPPDQQRIQDKEGIPPDQQRIQDKEGIPPDQQRDVSLVANHIDTVGKTAATVNTWTGGWSDSKAIGTYQNSGLSQYTVRYSEGVHFPARTVANWLVREVAGDVDNAVNPAWRLGAGVQGFEAYEAANAQGLRLDGGVIEDFAQKNPDLSSTSDTTDVIRGPDEPYSGQYDEERQFISVTNPTGAEPVPKFLSELLEDEYFTKFVNIWLENTDYESAANDPHLSKLLEYDIASGTPVYRNNNQGLEALTISPDGKVYAISDQDDTGPWIRDAYQNDFAARVDPSTAVDYNHYSDAADRSGDVQTLQFAWALQHLSERTGNQTGQLGTYFNKNINMLLYGTDDCSGKGMVFSIDAQGEKNINMLLYGTDDCSGKNPNPDQAFLQVRFWVATGDSSKAALDALQQSIYLQPKFSDGNGLFYQYERVAVAGYDDTTGGVGPLLAQKAIAIALQSSHRQTGSVDGYAYTDANKNDLITYLKSVVENNNDGLTAAYRVAPNSGAYLNEADFRSLPLIVGNSDQEGKANEQPTWVYRSDYQECADAPGQKFGATGDEYREPSNDPNPPETYSKVALLFSERLADGSIPTRSISSDEDSAETEQSDSSDPKVAIIDGLADPWRTMGVGYATNDDSTIRDVPIMQELNTNTIRDVDPIVIKVETGVIKPGMVVTFAPANVTTEVKIVVIGHVDSGKDDADLQELGAKSSAFAFRKDPSDAIPSIPSIPISYKEAIPFLKEAAEIDSHWERDDYMPFIEVPRDDYMPFIEVPRALQGVDELVEKDALHPQFDNFYQEQPKASYGAGVTIQDRDLSVFFTRINDLLPVYVELLQKAALTNMVNAAKGEITPEQYEKIINEPTAAAIAYGLDKQLTSEEIWQAEEKLDKPAGDYTIRDYSNNWESGALKLAPNQMTGSLDATYLKLAPNQMTGSLDATYLKCASDGSAETCSWEGHCKCASDGSAETCSWEGHCKCASDGSAETCSWEGHCKCASDGSAETCSWEGHCKCASDGSAETCSWEGHCKLAAISVEPGKASELGCSSGDLDCLCKVGECAQMCISNMNAKGTLLSSNQGSQAADVKNDDDFLNYGISSKAPSVITYDEATKYEAAGITVHKDDYLPFIDMPSEVTQIDAKIPMALDDWPTLSNMIFSGKDNFDTSSVTHRGYQINFLSNSAKDNIQGITKPAIRDNIQGITKPAIGPLGLSPKLQLWDTAGQERAEDYLLNPSPKNFGIGQDIQPKIDATTNPGMRQLGLAMLGNKLVIDGLKEVTEIPATADASRVNVDYTEVPRLAVNMVPFPRYCDLILGEWRDQIKDVLRIDYIGGGDLFRGSSPNVLYKSANWTPPEGIVRAASTGSMAEQYTKAATGTYASSTTVYKAENQAVAVGRALVEGSTFAKALYSSAATGTYASSTTVYKATGTYASSTTVYKATTVYGESIKAYADGYVQIVQTYAASTGSMAEQYTKDLTWSYAALLTANNRFNVDETAFTGAWGRGQSAQGASPGVVIASPSKIGADGQSAQGASPGVVIASPSKIGSLAITDVSLPFFKIQGISNPSGALSSGGLGEPKKYTVPSTCGVKPSGALSSGGLGEPKQAILNNIGADGQSAQGASPGVVIASPSKSDPDYFYTWTRSIYAINSGRTGTYASSTTVYKTVGSSCPYCDSQAPQVRVQNGAVTWESDPNRVQNGAVTWESDPNRKPDYFYTWTRYTVPSTCGVKSSAATGTYASSTTVYKGAVTWESDPNRIVGSISQLGSWNPSSATALSAVQSDVWRDINTVLGSIHTFDPQNIGADGQSAQGASPGVVIASPSKAASTGSMAEQYTKAENQAVAVGRAENQAVAVGRALVEGSTFAKALVEGSTFAKALYSSAATGTYASSTTVYKAYADGYVQIVQTYAASTGSMAEQYTKDLTWSYAALLTANNRDLTWSYAALLTANNRIQGISNPSGALSSGGLGEPKIQGISNPSGALSSGGLGEPKNIGADGQSAQGASPGVVIASPSKPDYFYTWTRQAILNNIGADGQSAQGASPGVVIASPSKQAILNNIGADGQSAQGASPGVVIASPSKQAILNNIGADGQSAQGASPGVVIASPSKQAILNNIGADGQSAQGASPGVVIASPSKQAILNNIGADGQSAQGASPGVVIASPSKQAILNNIGADGQSAQGASPGVVIASPSKQAILNNIGADGQSAQGASPGVVIASPSKQAILNNIGADGQSAQGASPGVVIASPSKQAILNNIGADGQSAQGASPGVVIASPSKQAILNNIGADGQSAQGASPGVVIASPSKQAILNNIGADGQSAQGASPGVVIASPSKQAILNNIGADGQSAQGASPGVVIASPSKQAILNNIGADGQSAQGASPGVVIASPSKSAVQSDVWRSAVQSDVWRSAVQSDVWRSAVQSDVWRSAVQSDVWRSDPDYFYTWTRSDPDYFYTWTRSDPDYFYTWTRSDPDYFYTWTRSDPDYFYTWTRSDPDYFYTWTRSIYAINSGRSIYAINSGRSIYAINSGRTVGSSCPYCDSQAPQVRTVGSSCPYCDSQAPQVRVQNGAVTWESDPNRVQNGAVTWESDPNRVQNGAVTWESDPNRVQNGAVTWESDPNRVQNGAVTWESDPNRVQNGAVTWESDPNRVQNGAVTWESDPNRVQNGAVTWESDPNRVQNGAVTWESDPNRVQNGAVTWESDPNRVQNGAVTWESDPNRVQNGAVTWESDPNRVQNGAVTWESDPNRVQNGAVTWESDPNRKVQNGAVTWESDPNRKVQNGAVTWESDPNRKVQNGAVTWESDPNRKASMVWEEAQQVSGKAVSPSFEDVWSQPRDGAGQMFIPLNPNAYSPNTLNKDVGGPIEDQNSLQVGDRFGFDLFDPTKGPTLLEDFIFRHGGPNFEQLPINQPRHVDGFGIHLFSYLDTQLNRLFYNSLTPAEQQFVVDAIRNNVIIQLNRQDLFEAIEAGRSLTPAEQQFVVDAIRSVTSGFVDGIKVGFLASVETPASIEAASELSKTTDVGTFGQKDVHGFATRIVPEEYVPITKFVTDNGDSKASMVWEEAQQVSGKASMVWEEAQQVSGKASMVWEEAQQVSGKASMVWEEAQQVSGKASMVWEEAQQVSGKASMVWEEAQQVSGKAVSPSFEDVWSQPRAVSPSFEDVWSQPRAVSPSFEDVWSQPRAVSPSFEDVWSQPRAVSPSFEDVWSQPRDGAGQMFIPLNPNAYSPNTLNKDGAGQMFIPLNPNAYSPNTLNKHGGPNFEQLPINQPRHGGPNFEQLPINQPRHGGPNFEQLPINQPRHGGPNFEQLPINQPRLFSYLDTQLNRNNVIIQLNRNNVIIQLNRNNVIIQLNRSVTSGFVDGIKSVTSGFVDGIKAAALAELVWSGNRAELVWSGNRASNSLQYVNVQVKDAYSPHEIYSREYLVANGVQAQALVPKGIMLDTGRGVQAQALVPKHIVGATAPLWGEQVDDINVSHIVGATAPLWGEQVDDINVSSMIFEQLEGMSLSKVIPEIDMPSHSSSGWKYNVMANPDANTPNFNYGGNGGSWCAPYKTYEVVGNVYKDIEADLQHAETVWGALHAFLVMWEDIALSADNAHDVPKAAALAELVWSGNRAAALAELVWSGNRAAALAELVWSGNRAAALAELVWSGNRASNSLQYVNVQVKASNSLQYVNVQVKASNSLQYVNVQVKASNSLQYVNVQVKDAYSPHEIYSRDAYSPHEIYSRDAYSPHEIYSRDAYSPHEIYSRDAYSPHEIYSRDAYSPHEIYSRDAYSPHEIYSREYLVANGVQAQALVPKEYLVANGVQAQALVPKEYLVANGVQAQALVPKGIMLDTGRIFEQLEGMSLSKIFEQLEGMSLSKIFEQLEGMSLSKIFEQLEGMSLSKTYEVVGNVYKYNVMANPDANTPNFNYGGNGGSWCAPYKYNVMANPDANTPNFNYGGNGGSWCAPYKYNVMANPDANTPNFNYGGNGGSWCAPYKYNVMANPDANTPNFNYGGNGGSWCAPYKATSGGTSAAAPVFAGLVGMLNDARAWYQESAVSKDFTDITAGSSIGCDGVNPQTGKGFPDVAAHSLTPRPDVAAHSLTPRPNSALPQVLSNSYGDEEQTVPEYYAKSALPQVLSNSYGDEEQTVPEYYAKSNSYGDEEQTVPEYYAKSYGDEEQTVPEYYAKYLDQQITAETKAWYQESAVSKAWYQESAVSKAWYQESAVSKAWYQESAVSKGFPDVAAHSLTPRGFPDVAAHSLTPRGFPDVAAHSLTPRGFPDVAAHSLTPRGFPDVAAHSLTPRPDVAAHSLTPRSALPQVLSNSYGDEEQTVPEYYAKYLDQQITAETKYLDQQITAETKANEQPTWVYRFFCPTDYLIDVRGTPSVLTEQGLVKLGVPGNELAIEIGSTGDYNARQGTPSVLTEQGLVKSLPLIVGNSDQEGKTFQGTPSVLTEQGLVKYPVVQNPVTLAESSCQSVFNPNIPKNPSAGPGWDQAKPTNGPLAKFQGTPSVLTEQGLVKANEQPTWVYRANEQPTWVYRGTPSVLTEQGLVKNPSAGPGWDQAKPTNGPLAKSLPLIVGNSDQEGKSLPLIVGNSDQEGKSLPLIVGNSDQEGKARNHGTSTVAPQVQASVYRASVDISNVDTYSSTEVANDDSFQQVGKATFLVWDQQRKASVDISNVDTYSSTEVANDDSFQQVGKNHGTSTVAPQVQASVYRSSTEVANDDSFQQVGKTLYLTDTDAGVPMIDPRTVYAFDVSEDGSYLKVASNGYVITGAGKARNHGTSTVAPQVQASVYRARNHGTSTVAPQVQASVYRATFLVWDQQRATFLVWDQQRATFLVWDQQRKASVDISNVDTYSSTEVANDDSFQQVGKTVYAFDVSEDGSYLKVASNGYVITGAGKVASNGYVITGAGKIENQSDADGYSSCSTLKLTGLTTLTTLSFAALTKSASSLNSIGDTFKSDKLNVIDFPKSLNSIGDTFKVGSIEFTALPQLQSLDFTKTVNGGFQIARLNVIDFPKGQLGFWGNKGTYSGDLQLNGVKLNVIDFPKSDKLNVIDFPKSDKLNVIDFPKTVNGGFQIARTVNGGFQIARAVGSDEWTVRLGITYTTYSKMTNDYISALTKSEMLAEQDKMTNDYISALTKSTITTPWKSVVENNNDGLTAAYRVAPNSGAYLNEADFRYFYGDNYATLRSGAYLNEADFRTAVGSDEWTVRLGITYTTYSKMTNDYISALTKMTNDYISALTKMTNDYISALTKSEMLAEQDKMTNDYISALTKSEMLAEQDKMTNDYISALTKSEMLAEQDKMTNDYISALTKSVVENNNDGLTAAYRSVVENNNDGLTAAYRSVVENNNDGLTAAYRSVVENNNDGLTAAYRETTMFVLQGFGASMARLNALQGGRLVQNDFNTLLRQDILGGMVDSYTDPKTGETTQIHARYGLEAAVPLMYESTGLGLGDMTKVSVADVKIDYIGGGDLFRLVQNDFNTLLRQDILGGMVDSYTDPKYGLEAAVPLMYESTGLGLGDMTKALEAYKVNGKAVDFSGHDEFQGKEPSNDPNPPETYSKFGATGDEYRSDYQECADAPGQKYIARPDIMKSTLPDLSEVIKVNGKEVGQFKSVDNFHLLTVYAVDFSGHDEFQGKFGATGDEYRYIARPDIMKFLDEALTYPPPKGIQINDPSINDDSVMIYAPAVRIASAMLDEEDEKYFNVKNGDQSPPSALGPLPSVIERPSINDDSVMIYAPAVRTDYSVCGETTIFKTVDDEEGVAAQFKIASAMLDEEDEKFLDEALTYPPPKFLDEALTYPPPKGIQINDPSINDDSVMIYAPAVRGIQINDPSINDDSVMIYAPAVRIASAMLDEEDEKIASAMLDEEDEKYFNVKIASAMLDEEDEKYFNVKNGDQSPPSALGPLPSVIERNGDQSPPSALGPLPSVIERAGAVAAVVYNNEKHGIPGGGIATGAEGIKLVLGDAVPESAAPMGLTPPTKSDKELVSSSAFQSHVKSFEGFPKRLVAHSVATYARIADLGKEEYNHPTRAGAVAAVVYNNEKHGIPGGGIATGAEGIKHGIPGGGIATGAEGIKLVLGDAVPESAAPMGLTPPTKLVLGDAVPESAAPMGLTPPTKLVLGDAVPESAAPMGLTPPTKSDKELVSSSAFQSHVKFTDTPVLYGPKKFTDTPVLYGPKMLDDAGIYLITDLSSPSESINRQQLSFVMNQWYEKYGAYSVCSPKSDGQCSDLLKWDVDLYSRLITDLSSPSESINRDLSSPSESINRKFTDTPVLYGPKKFTDTPVLYGPKQQLSFVMNQWYEKQQLSFVMNQWYEKCDVATTDVYYSGKGGTPDFGPGRSKYTAEGYEAATKVATIGSATFARYCASAQEDNATLQALLRYTAEGYEAATKYVDAGGFEPSIKSKYTAEGYEAATKVATIGSATFARVATIGSATFARYVDAGGFEPSIKDADACNGGGIEYDSPADTPLEFKDNTCNAPIPVSFPVAPTDTKEISFNQAWLRFAANGNYGSETTAAVINNFNGRITTADMDGISSWLPTINGKVIANGNVAGNILVIAKSDVSDFKEAGLKDADACNGGGIEYDSPADTPLEFKDADACNGGGIEYDSPADTPLEFKDADACNGGGIEYDSPADTPLEFKFAANGNYGSETTAAVINNFNGRANNYCSNQVEGPYSLYSGRVSIWTESYGGRYGPSFTAFFQEQNEKTVYDMAMEAWSKISYKEPGICETTPGVKSAGYAPLKPGGCKDQIIECRANNYCSNQVEGPYSLYSGRANNYCSNQVEGPYSLYSGRANNYCSNQVEGPYSLYSGRISYKEPGICETTPGVKVSIWTESYGGRAIMGAEEAAKTGGAMWPYRTLIPDVVGIFAGTPKFVTNMQAALLKALSEMILQSEKDYYASMLQQPKANFEVETPRGITGTSIARANFEVETPRDYYASMLQQPKFVTNMQAALLKFVTNMQAALLKTGGAMWPYRTGGAMWPYRAEDYLLNPSPKLSDLTGDTEYAQLSQKTDDQVSLFETTIRTDSGFAGLTNVNAANGGGRYDNQESFLFAEVLKITGQEIYRAEDYLLNPSPKTDDQVSLFETTIRAGFAGDDAPRQEYDESGPSIVHRSYELPDGQVITIGNERVAPEEHPVLLTEAPINPKDLTDYLMKIIAPPERSYELPDGQVITIGNERVAPEEHPVLLTEAPINPKALLFGAAGSAEDPVVVKNVGFPVVTVAEDAASSSIKVYATPDQDIEHGRAVEQSLDAIRQGLLTVEDRGPLNEGGLYAERLSGQDASAITWKLTGNLGGEDYQDKASPSYLTATPRALMNGAGAIKDAGYETSITDYWGRPTVYGFVPLEYVGSKTAFSDILAKTNTQVPDACTQCFQKMPMPLLVADGRTAFSDILAKAFPDVAAQGMNFAVYDKELYNIGDYQADANSGSKIAFASYLEEYARLETIGDTFKQGLQDITLGASIGCTGRAFPDVAAQGMNFAVYDKELYNIGDYQADANSGSKQGLQDITLGASIGCTGRLVEGAAAGIVVASPSKQGVLNNIGADGKSSSAYESLTSAVKASALIAYGNSLISSDKSVYGINNGRPDYFYTWTRPDYFYTWTRSNPDYFYTWTRSNPDYFYTWTRSNPDYFYTWTRSNPDYFYTWTRSNPDYFYTWTRSNPDYFYTWTRFSVAEILPGAKNVVLDTTALSANTKVGTIITGDPLDPPVLKYPAEVFLPGGTYQLGKADKETDIGSAIEKASAIQLDGIIYRQLSGHVGPLTSSSSKETDIGSAIEKADKETDIGSAIEKQLSGHVGPLTSSSSKQLSGHVGPLTSSSSKIYSFFVGGAVPENLRQTSSEQNPSLEEIQAAQATVLPHSPVSNVKSAGEYNTFSPEWPVPLTKTFDENDTYEIGNKSIDQFFNDAKVPTVLMSPWVGKDGQEATFHFDRVDWSPSFRAAEVINYYTPDHVPVFNAMSIDQFFNDAKNAFITNYPSEQRYDTATFIDKRIDATTNPGMRQLGLAMLGNKNMHDVIGNDGTVPSEFRIDATTNPGMRIDATTNPGMRNAFITNYPSEQRNAFITNYPSEQRQLGLAMLGNKAQITAVNLEARGDGGGGPTFEHLEKSMDNDNTSLLVFGKMGESVDDFFARAQITAVNLEARMGESVDDFFARGIVSGEGEESSDPVKVDNVVASFKYMQQLLDQTKVVWQDSVRAQNDPNAFGVVAARDPNAFGVVAARNDPNAFGVVAARAATYCPENIEKAQNDPNAFGVVAARAQNDPNAFGVVAARTIFGWDIAEGQKSAGYTPLKVNGVEYGETRSAGYTPLKVNGVEYGETRSAGYTPLKVNGVEYGETRGGSILPMQEVALTTRWASVIDATKKATGDVLFNTKHTADGAWAKGGSILPMQEVALTTRGGSILPMQEVALTTRWASVIDATKDGLEGSFKWDNLDSAALNTKVEDGNLILTMPKVEDGNLILTMPKVEDGNLILTMPKWDNLDSAALNTKWDNLDSAALNTKSAISQYGDSFAKSQSDFESEFSTAKVNAGIGIGPDDLVSFIKSAISQYGDSFAKSQSDFESEFSTAKGFNIVVAPGLDGRHVDVPLTGEDEITILAIHDEVSPVGDTDALLERAPVVQYALNRYLVDQLNPEGKAIHDEVSPVGDTDALLERAIHDEVSPVGDTDALLERAPVVQYALNRAPVVQYALNRDAELTDAGVKQAQVAHDFWQKLNTGAVIPVLVRLGDLSANPIERVLPQVIEATNRIYVTGQSYAGRLGDLSANPIERVLPQVIEATNRVLPQVIEATNRNDPVAVFDGSVIPKEAGLVPFQVSPTTKTLGIDIARGQTPLPILVADGRTSTTLPEVCSKNNILEGPDVKGQTPLPILVADGRINTAAYWKEAIADVLEHLGENDEDIAVYAPNPFYKNSILEGPDVKMPMPILVADGRMPMPILVADGRNDDDFLNYGISSKSPVTSEYTSVRSIFEAANEKAINDYIDSQLDKYLTNSQALADLPYFAEKGVQISTNIPKGVQISTNIPKEIISTYSIDGLRSVYQTMTDRYNTDAELYKGGSELGFRSAADGLASAITSKSGDDISTTDALALPEPVQALTKAGSSPTDIISGISDKTDALDSAIKYDYENVDSDGANKYNLSNGAPAPETVTNKSMPTSGAVDLVAKCSSHDDCSDELACTDGVCACTADSAVTCSWEGHCAGAKGDNPSILGLRCTADSAVTCSWEGHCAGAKDSPNWDVDSDALPAIPEGAKTLADFDALKTLADFDALKINPGPLARLYPDDNLAFIQAGISDEKLYTGEVFKTDEGKGQEPPAAIVEVQKVAIIDGLADPWRSVNIVNYTPSDSYTYSDNSGSWQSVKVTTGGQGAEFTLAKDQTTWSVDGNVVRVTTGGQGAEFTLAKVTTGGQGAEFTLAKAGQFPISANDGATSTKEAASAALAAGYKQTYTSCNPLKKTLNYADALDGENYPQTPSRVAVAGYDDTTGGVGPLLAQKINPSSGLLEPQTPLAVSPGSGPRVAVAGYDDTTGGVGPLLAQKTTGAFDESGPPLSQKNALQTMYDTQDKAALDALQQSIYLQPKFSDGNGLFYQYERLGAEVVTAGRIYAVADTQERLINQVELSEDKAVITDIVNQQRAVITDIVNQQRGENILSAPLITYAPAGPELDEKELGFTAVGGEGKDIQYLENYQGQGYSGPAVKILQYAQGRDYSNNWESGALKDDYMPFIEVPREAAEIDSHWERTIPIDNDVDYVVTGYRVYWVDSGPRTGDGVNDAPSLKDGQEQEILARADAIVAAIRSALIAFEKNINMLLYGTDDCSGKGMVFSIDAQGEKTGTDQASVGYYKDAVYALDAIYGIDARDNILPENLDDGLPSQFVYEKILVENLQDQTAKILVENLQDQTAKAEPYVTGSSAASGSNFVADFAEAGTDGKQISYWAFTTPAVKFEPPAVYNDELKDAEEEPYDWSNEGRLSDELEDDNAPIGFETTKDQEMAVAAFRTSDDFASQMDGRCMGCDSTSIDVSRCMGCDSTSIDVSRDASGGDQITEWQDIYLPPITKGIQDAGVIATAKGVGSDAWTVSESGRGIDGDKGLVVKDLYGNIVMSGGSTLYPGIADRAGFAGDDAPRQEYDESGPSIVHRSYELPDGQVITIGNERSYELPDGQVITIGNERLSGGVAVIKTTAVLFDEGKIGGSAGTELQSDKDLALVDPGLELSYNTKLVGGSDFGEDEAKTLSTNEEGYETSAVRASYGAGVTIQDRSAYVVYDLSNNEISLANTKVPYLIGANTDEGTSFAIRLPVEAFQALASSTSETKDAGNAATNDPLFPFSRAALPGTEVLFADSVAKVTSAQYYVNPKIQAFVIYPENFDKVGAGVNVGELYAFADKALTQYSVKTTYNVVAQTKTYANLPQALVNSGAIKVIPLQGCDADEYGRDNIQGITKPAIRLANAYTWEGGRYQGASQCPFRTMGVGYATNDDSTIRCASDGSAETCSWEGHCKCASDGSAETCSWEGHCKLILPGELAK